European Patent Application EP 4 595 966 A1, published August 6, 2025. Title: USE OF NPY/Y5R INHIBITOR IN TREATING LIVER METASTASIS. Applicant: Friedrich-Alexander-Universität Erlangen-Nürnberg. Application EP. The sequence listing filed with the application follows.

SEQUENCE LISTING (350 sequences)

SEQ ID NO: 1 - RNA, 21 nt, synthetic construct
  source 1..21: mol_type = other RNA
tctgggaacattttctgtgct

SEQ ID NO: 2 - RNA, 21 nt, synthetic construct
  source 1..21: mol_type = other RNA
tctgaaatcagtgtctctggg

SEQ ID NO: 3 - RNA, 21 nt, synthetic construct
  source 1..21: mol_type = other RNA
tcgttttccatatctctgcct

SEQ ID NO: 4 - RNA, 21 nt, synthetic construct
  source 1..21: mol_type = other RNA
ttctgtgctttctctcatcaa

SEQ ID NO: 5 - RNA, 21 nt, synthetic construct
  source 1..21: mol_type = other RNA
ttctgggaacattttctgtgc

SEQ ID NO: 6 - RNA, 21 nt, synthetic construct
  source 1..21: mol_type = other RNA
ttttccatatctctgcctggt

SEQ ID NO: 7 - RNA, 21 nt, synthetic construct
  source 1..21: mol_type = other RNA
ttgcagaattcagcacagtgg

SEQ ID NO: 8 - RNA, 21 nt, synthetic construct
  source 1..21: mol_type = other RNA
tcaagaggtctgaaatcagtg

SEQ ID NO: 9 - RNA, 21 nt, synthetic construct
  source 1..21: mol_type = other RNA
ttctctcatcaagaggtctga

SEQ ID NO: 10 - RNA, 21 nt, synthetic construct
  source 1..21: mol_type = other RNA
tgggaacattttctgtgcttt

SEQ ID NO: 11 - RNA, 21 nt, synthetic construct
  source 1..21: mol_type = other RNA
tttctgtgctttctctcatca

SEQ ID NO: 12 - RNA, 21 nt, synthetic construct
  source 1..21: mol_type = other RNA
tgaaaataggaaaaggccaga

SEQ ID NO: 13 - RNA, 21 nt, synthetic construct
  source 1..21: mol_type = other RNA
ttctcgttttacacgatgaaa

SEQ ID NO: 14 - RNA, 21 nt, synthetic construct
  source 1..21: mol_type = other RNA
tttctctcatcaagaggtctg

SEQ ID NO: 15 - RNA, 21 nt, synthetic construct
  source 1..21: mol_type = other RNA
aaataggaaaaggccagagag

SEQ ID NO: 16 - RNA, 21 nt, synthetic construct
  source 1..21: mol_type = other RNA
aataggaaaaggccagagagc

SEQ ID NO: 17 - RNA, 21 nt, synthetic construct
  source 1..21: mol_type = other RNA
atgaggttgatgtagtgtcgc

SEQ ID NO: 18 - RNA, 21 nt, synthetic construct
  source 1..21: mol_type = other RNA
aagtctcatttcccatcacca

SEQ ID NO: 19 - RNA, 21 nt, synthetic construct
  source 1..21: mol_type = other RNA
attctcgttttacacgatgaa

SEQ ID NO: 20 - RNA, 21 nt, synthetic construct
  source 1..21: mol_type = other RNA
atcaagaggtctgaaatcagt

SEQ ID NO: 21 - RNA, 21 nt, synthetic construct
  source 1..21: mol_type = other RNA
atttcccatcaccacattgca

SEQ ID NO: 22 - RNA, 21 nt, synthetic construct
  source 1..21: mol_type = other RNA
attttctgtgctttctctcat

SEQ ID NO: 23 - RNA, 21 nt, synthetic construct
  source 1..21: mol_type = other RNA
acattttctgtgctttctctc

SEQ ID NO: 24 - RNA, 21 nt, synthetic construct
  source 1..21: mol_type = other RNA
aaaacattgcagaattcagca

SEQ ID NO: 25 - RNA, 21 nt, synthetic construct
  source 1..21: mol_type = other RNA
aacattttctgtgctttctct

SEQ ID NO: 26 - RNA, 21 nt, synthetic construct
  source 1..21: mol_type = other RNA
atcgttttccatatctctgcc

SEQ ID NO: 27 - RNA, 21 nt, synthetic construct
  source 1..21: mol_type = other RNA
aagaggtctgaaatcagtgtc

SEQ ID NO: 28 - RNA, 21 nt, synthetic construct
  source 1..21: mol_type = other RNA
aaaataggaaaaggccagaga

SEQ ID NO: 29 - RNA, 21 nt, synthetic construct
  source 1..21: mol_type = other RNA
attgcagaattcagcacagtg

SEQ ID NO: 30 - RNA, 21 nt, synthetic construct
  source 1..21: mol_type = other RNA
tttcccatcaccacattgcag

SEQ ID NO: 31 - RNA, 21 nt, synthetic construct
  source 1..21: mol_type = other RNA
ttcaagccgagttctgggaac

SEQ ID NO: 32 - RNA, 21 nt, synthetic construct
  source 1..21: mol_type = other RNA
tatctggccatgtcctccgct

SEQ ID NO: 33 - RNA, 21 nt, synthetic construct
  source 1..21: mol_type = other RNA
tgatgtagtgtcgcagcgccg

SEQ ID NO: 34 - RNA, 21 nt, synthetic construct
  source 1..21: mol_type = other RNA
ttccatatctctgcctggtga

SEQ ID NO: 35 - RNA, 21 nt, synthetic construct
  source 1..21: mol_type = other RNA
tagtatctggccatgtcctcc

SEQ ID NO: 36 - RNA, 21 nt, synthetic construct
  source 1..21: mol_type = other RNA
taggatgggtggattctcgtt

SEQ ID NO: 37 - RNA, 21 nt, synthetic construct
  source 1..21: mol_type = other RNA
tcttcaagccgagttctggga

SEQ ID NO: 38 - RNA, 21 nt, synthetic construct
  source 1..21: mol_type = other RNA
ttgcagggtcttcaagccgag

SEQ ID NO: 39 - RNA, 21 nt, synthetic construct
  source 1..21: mol_type = other RNA
tctctgcctggtgatgaggtt

SEQ ID NO: 40 - RNA, 21 nt, synthetic construct
  source 1..21: mol_type = other RNA
ttgtccggcttggaggggtac

SEQ ID NO: 41 - RNA, 21 nt, synthetic construct
  source 1..21: mol_type = other RNA
tctggccatgtcctccgctgg

SEQ ID NO: 42 - RNA, 21 nt, synthetic construct
  source 1..21: mol_type = other RNA
tcgcccgggttgtccggcttg

SEQ ID NO: 43 - RNA, 21 nt, synthetic construct
  source 1..21: mol_type = other RNA
tcctcgcccgggttgtccggc

SEQ ID NO: 44 - RNA, 21 nt, synthetic construct
  source 1..21: mol_type = other RNA
tggtgcgtcctcgcccgggtt

SEQ ID NO: 45 - RNA, 21 nt, synthetic construct
  source 1..21: mol_type = other RNA
tctcatttcccatcaccacat

SEQ ID NO: 46 - RNA, 21 nt, synthetic construct
  source 1..21: mol_type = other RNA
ttcccatcaccacattgcagg

SEQ ID NO: 47 - RNA, 21 nt, synthetic construct
  source 1..21: mol_type = other RNA
tatctctgcctggtgatgagg

SEQ ID NO: 48 - RNA, 21 nt, synthetic construct
  source 1..21: mol_type = other RNA
tctctcatcaagaggtctgaa

SEQ ID NO: 49 - RNA, 21 nt, synthetic construct
  source 1..21: mol_type = other RNA
taggaaaaggccagagagcaa

SEQ ID NO: 50 - RNA, 21 nt, synthetic construct
  source 1..21: mol_type = other RNA
tttccatatctctgcctggtg

SEQ ID NO: 51 - RNA, 21 nt, synthetic construct
  source 1..21: mol_type = other RNA
tgaggttgatgtagtgtcgca

SEQ ID NO: 52 - RNA, 21 nt, synthetic construct
  source 1..21: mol_type = other RNA
ttgatgtagtgtcgcagcgcc

SEQ ID NO: 53 - RNA, 21 nt, synthetic construct
  source 1..21: mol_type = other RNA
agtggctgcatgcattggtag

SEQ ID NO: 54 - RNA, 21 nt, synthetic construct
  source 1..21: mol_type = other RNA
agtctcatttcccatcaccac

SEQ ID NO: 55 - RNA, 21 nt, synthetic construct
  source 1..21: mol_type = other RNA
agtagtatctggccatgtcct

SEQ ID NO: 56 - RNA, 21 nt, synthetic construct
  source 1..21: mol_type = other RNA
attgcagggtcttcaagccga

SEQ ID NO: 57 - RNA, 21 nt, synthetic construct
  source 1..21: mol_type = other RNA
atctggccatgtcctccgctg

SEQ ID NO: 58 - RNA, 21 nt, synthetic construct
  source 1..21: mol_type = other RNA
acacgagcagggacagggcga

SEQ ID NO: 59 - RNA, 21 nt, synthetic construct
  source 1..21: mol_type = other RNA
acagggcgagggtcagtccgg

SEQ ID NO: 60 - RNA, 21 nt, synthetic construct
  source 1..21: mol_type = other RNA
agggtcagtccggacagcccc

SEQ ID NO: 61 - RNA, 21 nt, synthetic construct
  source 1..21: mol_type = other RNA
aaatcagtgtctctgggctgg

SEQ ID NO: 62 - RNA, 21 nt, synthetic construct
  source 1..21: mol_type = other RNA
ataggaaaaggccagagagca

SEQ ID NO: 63 - RNA, 21 nt, synthetic construct
  source 1..21: mol_type = other RNA
aaggccagagagcaagtctca

SEQ ID NO: 64 - RNA, 21 nt, synthetic construct
  source 1..21: mol_type = other RNA
aggaaaaggccagagagcaag

SEQ ID NO: 65 - RNA, 21 nt, synthetic construct
  source 1..21: mol_type = other RNA
atgcattggtaggatgggtgg

SEQ ID NO: 66 - RNA, 21 nt, synthetic construct
  source 1..21: mol_type = other RNA
attggtaggatgggtggattc

SEQ ID NO: 67 - RNA, 21 nt, synthetic construct
  source 1..21: mol_type = other RNA
aattcagcacagtggctgcat

SEQ ID NO: 68 - RNA, 21 nt, synthetic construct
  source 1..21: mol_type = other RNA
agaattcagcacagtggctgc

SEQ ID NO: 69 - RNA, 21 nt, synthetic construct
  source 1..21: mol_type = other RNA
atatctctgcctggtgatgag

SEQ ID NO: 70 - RNA, 21 nt, synthetic construct
  source 1..21: mol_type = other RNA
aggttgatgtagtgtcgcagc

SEQ ID NO: 71 - RNA, 21 nt, synthetic construct
  source 1..21: mol_type = other RNA
atctctgcctggtgatgaggt

SEQ ID NO: 72 - RNA, 21 nt, synthetic construct
  source 1..21: mol_type = other RNA
aagccgagttctgggaacatt

SEQ ID NO: 73 - RNA, 21 nt, synthetic construct
  source 1..21: mol_type = other RNA
agggcgagggtcagtccggac

SEQ ID NO: 74 - RNA, 21 nt, synthetic construct
  source 1..21: mol_type = other RNA
agtatctggccatgtcctccg

SEQ ID NO: 75 - RNA, 21 nt, synthetic construct
  source 1..21: mol_type = other RNA
tcatttcccatcaccacattg

SEQ ID NO: 76 - RNA, 21 nt, synthetic construct
  source 1..21: mol_type = other RNA
tcgttttacacgatgaaatat

SEQ ID NO: 77 - RNA, 21 nt, synthetic construct
  source 1..21: mol_type = other RNA
tcatcaagaggtctgaaatca

SEQ ID NO: 78 - RNA, 21 nt, synthetic construct
  source 1..21: mol_type = other RNA
tctcatcaagaggtctgaaat

SEQ ID NO: 79 - RNA, 21 nt, synthetic construct
  source 1..21: mol_type = other RNA
tggattctcgttttacacgat

SEQ ID NO: 80 - RNA, 21 nt, synthetic construct
  source 1..21: mol_type = other RNA
tgtgctttctctcatcaagag

SEQ ID NO: 81 - RNA, 21 nt, synthetic construct
  source 1..21: mol_type = other RNA
tctcgttttacacgatgaaat

SEQ ID NO: 82 - RNA, 21 nt, synthetic construct
  source 1..21: mol_type = other RNA
tgggtggattctcgttttaca

SEQ ID NO: 83 - RNA, 21 nt, synthetic construct
  source 1..21: mol_type = other RNA
agaggtctgaaatcagtgtct

SEQ ID NO: 84 - RNA, 21 nt, synthetic construct
  source 1..21: mol_type = other RNA
atgggtggattctcgttttac

SEQ ID NO: 85 - RNA, 21 nt, synthetic construct
  source 1..21: mol_type = other RNA
agcaagtctcatttcccatca

SEQ ID NO: 86 - RNA, 21 nt, synthetic construct
  source 1..21: mol_type = other RNA
aggtctgaaatcagtgtctct

SEQ ID NO: 87 - RNA, 21 nt, synthetic construct
  source 1..21: mol_type = other RNA
tgcattggtaggatgggtgga

SEQ ID NO: 88 - RNA, 21 nt, synthetic construct
  source 1..21: mol_type = other RNA
tgcagaattcagcacagtggc

SEQ ID NO: 89 - RNA, 21 nt, synthetic construct
  source 1..21: mol_type = other RNA
ttggtaggatgggtggattct

SEQ ID NO: 90 - RNA, 21 nt, synthetic construct
  source 1..21: mol_type = other RNA
tgcatgcattggtaggatggg

SEQ ID NO: 91 - RNA, 21 nt, synthetic construct
  source 1..21: mol_type = other RNA
tcaagccgagttctgggaaca

SEQ ID NO: 92 - RNA, 21 nt, synthetic construct
  source 1..21: mol_type = other RNA
tcccatcaccacattgcaggg

SEQ ID NO: 93 - RNA, 21 nt, synthetic construct
  source 1..21: mol_type = other RNA
tggctgcatgcattggtagga

SEQ ID NO: 94 - RNA, 21 nt, synthetic construct
  source 1..21: mol_type = other RNA
tgcagggtcttcaagccgagt

SEQ ID NO: 95 - RNA, 21 nt, synthetic construct
  source 1..21: mol_type = other RNA
tcctccgctggtgcgtcctcg

SEQ ID NO: 96 - RNA, 21 nt, synthetic construct
  source 1..21: mol_type = other RNA
tccatatctctgcctggtgat

SEQ ID NO: 97 - RNA, 21 nt, synthetic construct
  source 1..21: mol_type = other RNA
tggccatgtcctccgctggtg

SEQ ID NO: 98 - RNA, 21 nt, synthetic construct
  source 1..21: mol_type = other RNA
tgcctggtgatgaggttgatg

SEQ ID NO: 99 - RNA, 21 nt, synthetic construct
  source 1..21: mol_type = other RNA
tggtaggatgggtggattctc

SEQ ID NO: 100 - RNA, 21 nt, synthetic construct
  source 1..21: mol_type = other RNA
tcaccacattgcagggtcttc

SEQ ID NO: 101 - RNA, 21 nt, synthetic construct
  source 1..21: mol_type = other RNA
tgtccggcttggaggggtacg

SEQ ID NO: 102 - RNA, 21 nt, synthetic construct
  source 1..21: mol_type = other RNA
tgcgtcctcgcccgggttgtc

SEQ ID NO: 103 - RNA, 21 nt, synthetic construct
  source 1..21: mol_type = other RNA
tctgcctggtgatgaggttga

SEQ ID NO: 104 - RNA, 21 nt, synthetic construct
  source 1..21: mol_type = other RNA
aggccagagagcaagtctcat

SEQ ID NO: 105 - RNA, 21 nt, synthetic construct
  source 1..21: mol_type = other RNA
agcgcacccaggcacacgagc

SEQ ID NO: 106 - RNA, 21 nt, synthetic construct
  source 1..21: mol_type = other RNA
agggtcttcaagccgagttct

SEQ ID NO: 107 - RNA, 21 nt, synthetic construct
  source 1..21: mol_type = other RNA
aggatgggtggattctcgttt

SEQ ID NO: 108 - RNA, 21 nt, synthetic construct
  source 1..21: mol_type = other RNA
agcacagtggctgcatgcatt

SEQ ID NO: 109 - RNA, 21 nt, synthetic construct
  source 1..21: mol_type = other RNA
acccaggcacacgagcaggga

SEQ ID NO: 110 - RNA, 21 nt, synthetic construct
  source 1..21: mol_type = other RNA
aggcacacgagcagggacagg

SEQ ID NO: 111 - RNA, 21 nt, synthetic construct
  source 1..21: mol_type = other RNA
acagtggctgcatgcattggt

SEQ ID NO: 112 - RNA, 21 nt, synthetic construct
  source 1..21: mol_type = other RNA
agccgagttctgggaacattt

SEQ ID NO: 113 - RNA, 21 nt, synthetic construct
  source 1..21: mol_type = other RNA
accacattgcagggtcttcaa

SEQ ID NO: 114 - RNA, 21 nt, synthetic construct
  source 1..21: mol_type = other RNA
tacacgatgaaatatgggctg

SEQ ID NO: 115 - RNA, 21 nt, synthetic construct
  source 1..21: mol_type = other RNA
ttttacacgatgaaatatggg

SEQ ID NO: 116 - RNA, 21 nt, synthetic construct
  source 1..21: mol_type = other RNA
tatgggctgaaaataggaaaa

SEQ ID NO: 117 - RNA, 21 nt, synthetic construct
  source 1..21: mol_type = other RNA
tttacacgatgaaatatgggc

SEQ ID NO: 118 - RNA, 21 nt, synthetic construct
  source 1..21: mol_type = other RNA
ttacacgatgaaatatgggct

SEQ ID NO: 119 - RNA, 21 nt, synthetic construct
  source 1..21: mol_type = other RNA
acacgatgaaatatgggctga

SEQ ID NO: 120 - RNA, 21 nt, synthetic construct
  source 1..21: mol_type = other RNA
aaatatgggctgaaaatagga

SEQ ID NO: 121 - RNA, 21 nt, synthetic construct
  source 1..21: mol_type = other RNA
aatatgggctgaaaataggaa

SEQ ID NO: 122 - RNA, 21 nt, synthetic construct
  source 1..21: mol_type = other RNA
atatgggctgaaaataggaaa

SEQ ID NO: 123 - RNA, 21 nt, synthetic construct
  source 1..21: mol_type = other RNA
tggaggggtacgcctcggcca

SEQ ID NO: 124 - RNA, 21 nt, synthetic construct
  source 1..21: mol_type = other RNA
tagtgtcgcagcgccgagtag

SEQ ID NO: 125 - RNA, 21 nt, synthetic construct
  source 1..21: mol_type = other RNA
tcagtccggacagccccagtc

SEQ ID NO: 126 - RNA, 21 nt, synthetic construct
  source 1..21: mol_type = other RNA
tccggacagccccagtcgctt

SEQ ID NO: 127 - RNA, 21 nt, synthetic construct
  source 1..21: mol_type = other RNA
tgtagtgtcgcagcgccgagt

SEQ ID NO: 128 - RNA, 21 nt, synthetic construct
  source 1..21: mol_type = other RNA
ttggaggggtacgcctcggcc

SEQ ID NO: 129 - RNA, 21 nt, synthetic construct
  source 1..21: mol_type = other RNA
tacgcctcggccagcgcaccc

SEQ ID NO: 130 - RNA, 21 nt, synthetic construct
  source 1..21: mol_type = other RNA
tgtctctgggctggatcgttt

SEQ ID NO: 131 - RNA, 21 nt, synthetic construct
  source 1..21: mol_type = other RNA
agtccggacagccccagtcgc

SEQ ID NO: 132 - RNA, 21 nt, synthetic construct
  source 1..21: mol_type = other RNA
acgcctcggccagcgcaccca

SEQ ID NO: 133 - RNA, 21 nt, synthetic construct
  source 1..21: mol_type = other RNA
agtcgcttgttacctagcatg

SEQ ID NO: 134 - RNA, 21 nt, synthetic construct
  source 1..21: mol_type = other RNA
aatcagtgtctctgggctgga

SEQ ID NO: 135 - RNA, 21 nt, synthetic construct
  source 1..21: mol_type = other RNA
atgtagtgtcgcagcgccgag

SEQ ID NO: 136 - RNA, 21 nt, synthetic construct
  source 1..21: mol_type = other RNA
tggatcgttttccatatctct

SEQ ID NO: 137 - RNA, 21 nt, synthetic construct
  source 1..21: mol_type = other RNA
tgggctgaaaataggaaaagg

SEQ ID NO: 138 - RNA, 21 nt, synthetic construct
  source 1..21: mol_type = other RNA
tgaaatatgggctgaaaatag

SEQ ID NO: 139 - RNA, 21 nt, synthetic construct
  source 1..21: mol_type = other RNA
atgggctgaaaataggaaaag

SEQ ID NO: 140 - RNA, 21 nt, synthetic construct
  source 1..21: mol_type = other RNA
atgaaatatgggctgaaaata

SEQ ID NO: 141 - RNA, 21 nt, synthetic construct
  source 1..21: mol_type = other RNA
acgatgaaatatgggctgaaa

SEQ ID NO: 142 - RNA, 21 nt, synthetic construct
  source 1..21: mol_type = other RNA
tgggctggatcgttttccata

SEQ ID NO: 143 - RNA, 21 nt, synthetic construct
  source 1..21: mol_type = other RNA
tctctgggctggatcgttttc

SEQ ID NO: 144 - RNA, 21 nt, synthetic construct
  source 1..21: mol_type = other RNA
tcgcagcgccgagtagtatct

SEQ ID NO: 145 - RNA, 21 nt, synthetic construct
  source 1..21: mol_type = other RNA
tgtcgcagcgccgagtagtat

SEQ ID NO: 146 - RNA, 21 nt, synthetic construct
  source 1..21: mol_type = other RNA
tctgggctggatcgttttcca

SEQ ID NO: 147 - RNA, 21 nt, synthetic construct
  source 1..21: mol_type = other RNA
tccggcttggaggggtacgcc

SEQ ID NO: 148 - RNA, 21 nt, synthetic construct
  source 1..21: mol_type = other RNA
agccccagtcgcttgttacct

SEQ ID NO: 149 - RNA, 21 nt, synthetic construct
  source 1..21: mol_type = other RNA
agcgccgagtagtatctggcc

SEQ ID NO: 150 - RNA, 21 nt, synthetic construct
  source 1..21: mol_type = other RNA
acagccccagtcgcttgttac

SEQ ID NO: 151 - RNA, 21 nt, synthetic construct
  source 1..21: mol_type = other RNA
agtgtcgcagcgccgagtagt

SEQ ID NO: 152 - RNA, 21 nt, synthetic construct
  source 1..21: mol_type = other RNA
agtgtctctgggctggatcgt

SEQ ID NO: 153 - RNA, 21 nt, synthetic construct
  source 1..21: mol_type = other RNA
aggggtacgcctcggccagcg

SEQ ID NO: 154 - RNA, 21 nt, synthetic construct
  source 1..21: mol_type = other RNA
tgacaaaggaaaacattgcag

SEQ ID NO: 155 - RNA, 21 nt, synthetic construct
  source 1..21: mol_type = other RNA
atatatacaatgatgacaaag

SEQ ID NO: 156 - RNA, 21 nt, synthetic construct
  source 1..21: mol_type = other RNA
atgatgacaaaggaaaacatt

SEQ ID NO: 157 - RNA, 21 nt, synthetic construct
  source 1..21: mol_type = other RNA
acaaaggaaaacattgcagaa

SEQ ID NO: 158 - RNA, 21 nt, synthetic construct
  source 1..21: mol_type = other RNA
atatacaatgatgacaaagga

SEQ ID NO: 159 - RNA, 21 nt, synthetic construct
  source 1..21: mol_type = other RNA
atacaatgatgacaaaggaaa

SEQ ID NO: 160 - RNA, 21 nt, synthetic construct
  source 1..21: mol_type = other RNA
aatgatgacaaaggaaaacat

SEQ ID NO: 161 - RNA, 21 nt, synthetic construct
  source 1..21: mol_type = other RNA
acatatatacaatgatgacaa

SEQ ID NO: 162 - RNA, 21 nt, synthetic construct
  source 1..21: mol_type = other RNA
aaaggaaaacattgcagaatt

SEQ ID NO: 163 - RNA, 21 nt, synthetic construct
  source 1..21: mol_type = other RNA
tgggcggcaagtactatgctg

SEQ ID NO: 164 - RNA, 21 nt, synthetic construct
  source 1..21: mol_type = other RNA
ttgttacctagcatggtggct

SEQ ID NO: 165 - RNA, 21 nt, synthetic construct
  source 1..21: mol_type = other RNA
ttacctagcatggtggctggc

SEQ ID NO: 166 - RNA, 21 nt, synthetic construct
  source 1..21: mol_type = other RNA
tgtcgggcgagcgtctccgag

SEQ ID NO: 167 - RNA, 21 nt, synthetic construct
  source 1..21: mol_type = other RNA
tctccgaggggtgagagccag

SEQ ID NO: 168 - RNA, 21 nt, synthetic construct
  source 1..21: mol_type = other RNA
tcgggcgagcgtctccgaggg

SEQ ID NO: 169 - RNA, 21 nt, synthetic construct
  source 1..21: mol_type = other RNA
tgttacctagcatggtggctg

SEQ ID NO: 170 - RNA, 21 nt, synthetic construct
  source 1..21: mol_type = other RNA
tggtggctggcgcgcgggcgt

SEQ ID NO: 171 - RNA, 21 nt, synthetic construct
  source 1..21: mol_type = other RNA
tacctagcatggtggctggcg

SEQ ID NO: 172 - RNA, 21 nt, synthetic construct
  source 1..21: mol_type = other RNA
tactatgctgtcgggcgagcg

SEQ ID NO: 173 - RNA, 21 nt, synthetic construct
  source 1..21: mol_type = other RNA
tatgctgtcgggcgagcgtct

SEQ ID NO: 174 - RNA, 21 nt, synthetic construct
  source 1..21: mol_type = other RNA
tagcatggtggctggcgcgcg

SEQ ID NO: 175 - RNA, 21 nt, synthetic construct
  source 1..21: mol_type = other RNA
agtactatgctgtcgggcgag

SEQ ID NO: 176 - RNA, 21 nt, synthetic construct
  source 1..21: mol_type = other RNA
atggtggctggcgcgcgggcg

SEQ ID NO: 177 - RNA, 21 nt, synthetic construct
  source 1..21: mol_type = other RNA
aagtactatgctgtcgggcga

SEQ ID NO: 178 - RNA, 21 nt, synthetic construct
  source 1..21: mol_type = other RNA
atgctgtcgggcgagcgtctc

SEQ ID NO: 179 - RNA, 21 nt, synthetic construct
  source 1..21: mol_type = other RNA
actatgctgtcgggcgagcgt

SEQ ID NO: 180 - RNA, 21 nt, synthetic construct
  source 1..21: mol_type = other RNA
tgatgacaaaggaaaacattg

SEQ ID NO: 181 - RNA, 21 nt, synthetic construct
  source 1..21: mol_type = other RNA
tgcatgatactttatttaaac

SEQ ID NO: 182 - RNA, 21 nt, synthetic construct
  source 1..21: mol_type = other RNA
ttgaatgcatgatactttatt

SEQ ID NO: 183 - RNA, 21 nt, synthetic construct
  source 1..21: mol_type = other RNA
tgaatgcatgatactttattt

SEQ ID NO: 184 - RNA, 21 nt, synthetic construct
  source 1..21: mol_type = other RNA
tacaatgatgacaaaggaaaa

SEQ ID NO: 185 - RNA, 21 nt, synthetic construct
  source 1..21: mol_type = other RNA
tatatacaatgatgacaaagg

SEQ ID NO: 186 - RNA, 21 nt, synthetic construct
  source 1..21: mol_type = other RNA
acaatgatgacaaaggaaaac

SEQ ID NO: 187 - RNA, 21 nt, synthetic construct
  source 1..21: mol_type = other RNA
aatgcatgatactttatttaa

SEQ ID NO: 188 - RNA, 21 nt, synthetic construct
  source 1..21: mol_type = other RNA
tcgcttgttacctagcatggt

SEQ ID NO: 189 - RNA, 21 nt, synthetic construct
  source 1..21: mol_type = other RNA
tggctgggcggcaagtactat

SEQ ID NO: 190 - RNA, 21 nt, synthetic construct
  source 1..21: mol_type = other RNA
tccgaggggtgagagccagcg

SEQ ID NO: 191 - RNA, 21 nt, synthetic construct
  source 1..21: mol_type = other RNA
tgctgtcgggcgagcgtctcc

SEQ ID NO: 192 - RNA, 21 nt, synthetic construct
  source 1..21: mol_type = other RNA
tggctggcgcgcgggcgtggc

SEQ ID NO: 193 - RNA, 21 nt, synthetic construct
  source 1..21: mol_type = other RNA
agcgtctccgaggggtgagag

SEQ ID NO: 194 - RNA, 21 nt, synthetic construct
  source 1..21: mol_type = other RNA
ttttctgtgctttctctcatc

SEQ ID NO: 195 - RNA, 21 nt, synthetic construct
  source 1..21: mol_type = other RNA
tgatgaggttgatgtagtgtc

SEQ ID NO: 196 - RNA, 21 nt, synthetic construct
  source 1..21: mol_type = other RNA
acattgcagaattcagcacag

SEQ ID NO: 197 - RNA, 21 nt, synthetic construct
  source 1..21: mol_type = other RNA
agttctgggaacattttctgt

SEQ ID NO: 198 - RNA, 21 nt, synthetic construct
  source 1..21: mol_type = other RNA
aaacattgcagaattcagcac

SEQ ID NO: 199 - RNA, 21 nt, synthetic construct
  source 1..21: mol_type = other RNA
aacattgcagaattcagcaca

SEQ ID NO: 200 - RNA, 21 nt, synthetic construct
  source 1..21: mol_type = other RNA
tgtcctccgctggtgcgtcct

SEQ ID NO: 201 - RNA, 21 nt, synthetic construct
  source 1..21: mol_type = other RNA
tccgctggtgcgtcctcgccc

SEQ ID NO: 202 - RNA, 21 nt, synthetic construct
  source 1..21: mol_type = other RNA
tcggccagcgcacccaggcac

SEQ ID NO: 203 - RNA, 21 nt, synthetic construct
  source 1..21: mol_type = other RNA
tgaaatcagtgtctctgggct

SEQ ID NO: 204 - RNA, 21 nt, synthetic construct
  source 1..21: mol_type = other RNA
aaaggccagagagcaagtctc

SEQ ID NO: 205 - RNA, 21 nt, synthetic construct
  source 1..21: mol_type = other RNA
agcagggacagggcgagggtc

SEQ ID NO: 206 - RNA, 21 nt, synthetic construct
  source 1..21: mol_type = other RNA
agagcaagtctcatttcccat

SEQ ID NO: 207 - RNA, 21 nt, synthetic construct
  source 1..21: mol_type = other RNA
atcaccacattgcagggtctt

SEQ ID NO: 208 - RNA, 21 nt, synthetic construct
  source 1..21: mol_type = other RNA
attcagcacagtggctgcatg

SEQ ID NO: 209 - RNA, 21 nt, synthetic construct
  source 1..21: mol_type = other RNA
aaaaggccagagagcaagtct

SEQ ID NO: 210 - RNA, 21 nt, synthetic construct
  source 1..21: mol_type = other RNA
acgagcagggacagggcgagg

SEQ ID NO: 211 - RNA, 21 nt, synthetic construct
  source 1..21: mol_type = other RNA
atgtcctccgctggtgcgtcc

SEQ ID NO: 212 - RNA, 21 nt, synthetic construct
  source 1..21: mol_type = other RNA
tctgtgctttctctcatcaag

SEQ ID NO: 213 - RNA, 21 nt, synthetic construct
  source 1..21: mol_type = other RNA
tgctttctctcatcaagaggt

SEQ ID NO: 214 - RNA, 21 nt, synthetic construct
  source 1..21: mol_type = other RNA
tggtgatgaggttgatgtagt

SEQ ID NO: 215 - RNA, 21 nt, synthetic construct
  source 1..21: mol_type = other RNA
agagagcaagtctcatttccc

SEQ ID NO: 216 - RNA, 21 nt, synthetic construct
  source 1..21: mol_type = other RNA
ttcagcacagtggctgcatgc

SEQ ID NO: 217 - RNA, 21 nt, synthetic construct
  source 1..21: mol_type = other RNA
tcagcacagtggctgcatgca

SEQ ID NO: 218 - RNA, 21 nt, synthetic construct
  source 1..21: mol_type = other RNA
acattgcagggtcttcaagcc

SEQ ID NO: 219 - RNA, 21 nt, synthetic construct
  source 1..21: mol_type = other RNA
agggacagggcgagggtcagt

SEQ ID NO: 220 - RNA, 21 nt, synthetic construct
  source 1..21: mol_type = other RNA
tcagtgtctctgggctggatc

SEQ ID NO: 221 - RNA, 21 nt, synthetic construct
  source 1..21: mol_type = other RNA
atcagtgtctctgggctggat

SEQ ID NO: 222 - RNA, 21 nt, synthetic construct
  source 1..21: mol_type = other RNA
tatacaatgatgacaaaggaa

SEQ ID NO: 223 - RNA, 21 nt, synthetic construct
  source 1..21: mol_type = other RNA
ttttgaatgcatgatacttta

SEQ ID NO: 224 - RNA, 21 nt, synthetic construct
  source 1..21: mol_type = other RNA
aggggtgagagccagcggatg

SEQ ID NO: 225 - RNA, 21 nt, synthetic construct
  source 1..21: mol_type = other RNA
acctagcatggtggctggcgc

SEQ ID NO: 226 - RNA, 21 nt, synthetic construct
  source 1..21: mol_type = other RNA
agcatggtggctggcgcgcgg

SEQ ID NO: 227 - RNA, 21 nt, synthetic construct
  source 1..21: mol_type = other RNA
tttgaatgcatgatactttat

SEQ ID NO: 228 - RNA, 21 nt, synthetic construct
  source 1..21: mol_type = other RNA
atgcatgatactttatttaaa

SEQ ID NO: 229 - RNA, 21 nt, synthetic construct
  source 1..21: mol_type = other RNA
aaggaaaacattgcagaattc

SEQ ID NO: 230 - RNA, 21 nt, synthetic construct
  source 1..21: mol_type = other RNA
atgacaaaggaaaacattgca

SEQ ID NO: 231 - RNA, 21 nt, synthetic construct
  source 1..21: mol_type = other RNA
aggaaaacattgcagaattca

SEQ ID NO: 232 - RNA, 21 nt, synthetic construct
  source 1..21: mol_type = other RNA
tggcgcgcgggcgtggctggg

SEQ ID NO: 233 - RNA, 19 nt, synthetic construct
  source 1..19: mol_type = other RNA
tgtcctctgctggcgcgtc

SEQ ID NO: 234 - RNA, 19 nt, synthetic construct
  source 1..19: mol_type = other RNA
atcaccacatggaagggtc

SEQ ID NO: 235 - RNA, 19 nt, synthetic construct
  source 1..19: mol_type = other RNA
ttaagaggtctgaaatcag

SEQ ID NO: 236 - RNA, 19 nt, synthetic construct
  source 1..19: mol_type = other RNA
acacgagcagagatagagc

SEQ ID NO: 237 - RNA, 19 nt, synthetic construct
  source 1..19: mol_type = other RNA
tttccttcattaagaggtc

SEQ ID NO: 238 - RNA, 19 nt, synthetic construct
  source 1..19: mol_type = other RNA
agcggagtagtatctggcc

SEQ ID NO: 239 - RNA, 19 nt, synthetic construct
  source 1..19: mol_type = other RNA
tcttcaagccttgttctgg

SEQ ID NO: 240 - RNA, 19 nt, synthetic construct
  source 1..19: mol_type = other RNA
tttcatttcccatcaccac

SEQ ID NO: 241 - RNA, 19 nt, synthetic construct
  source 1..19: mol_type = other RNA
atctcttgccatatctctg

SEQ ID NO: 242 - RNA, 19 nt, synthetic construct
  source 1..19: mol_type = other RNA
atggaagggtcttcaagcc

SEQ ID NO: 243 - RNA, 19 nt, synthetic construct
  source 1..19: mol_type = other RNA
tgatgagattgatgtagtg

SEQ ID NO: 244 - RNA, 19 nt, synthetic construct
  source 1..19: mol_type = other RNA
tgatgtagtgtcgcagagc

SEQ ID NO: 245 - RNA, 19 nt, synthetic construct
  source 1..19: mol_type = other RNA
tcctcgcccggattgtccg

SEQ ID NO: 246 - RNA, 19 nt, synthetic construct
  source 1..19: mol_type = other RNA
tcagggctggatctcttgc

SEQ ID NO: 247 - RNA, 19 nt, synthetic construct
  source 1..19: mol_type = other RNA
tctgaaatcagtgtctcag

SEQ ID NO: 248 - RNA, 19 nt, synthetic construct
  source 1..19: mol_type = other RNA
acaacaacaagggaaatgg

SEQ ID NO: 249 - RNA, 19 nt, synthetic construct
  source 1..19: mol_type = other RNA
tagtggtggcatgcattgg

SEQ ID NO: 250 - RNA, 19 nt, synthetic construct
  source 1..19: mol_type = other RNA
tgtctcagggctggatctc

SEQ ID NO: 251 - RNA, 19 nt, synthetic construct
  source 1..19: mol_type = other RNA
agagcggagtagtatctgg

SEQ ID NO: 252 - RNA, 19 nt, synthetic construct
  source 1..19: mol_type = other RNA
tgagattgatgtagtgtcg

SEQ ID NO: 253 - RNA, 19 nt, synthetic construct
  source 1..19: mol_type = other RNA
atagagcgagggtcagtcc

SEQ ID NO: 254 - RNA, 19 nt, synthetic construct
  source 1..19: mol_type = other RNA
ttgatgtagtgtcgcagag

SEQ ID NO: 255 - RNA, 19 nt, synthetic construct
  source 1..19: mol_type = other RNA
ttggaaaagtcgggagaac

SEQ ID NO: 256 - RNA, 19 nt, synthetic construct
  source 1..19: mol_type = other RNA
tgaaatcagtgtctcaggg

SEQ ID NO: 257 - RNA, 19 nt, synthetic construct
  source 1..19: mol_type = other RNA
atatctctgtctggtgatg

SEQ ID NO: 258 - RNA, 19 nt, synthetic construct
  source 1..19: mol_type = other RNA
aagaggtctgaaatcagtg

SEQ ID NO: 259 - RNA, 19 nt, synthetic construct
  source 1..19: mol_type = other RNA
atttcccatcaccacatgg

SEQ ID NO: 260 - RNA, 19 nt, synthetic construct
  source 1..19: mol_type = other RNA
agcagagatagagcgaggg

SEQ ID NO: 261 - RNA, 19 nt, synthetic construct
  source 1..19: mol_type = other RNA
aagtttcatttcccatcac

SEQ ID NO: 262 - RNA, 19 nt, synthetic construct
  source 1..19: mol_type = other RNA
agtagtatctggccatgtc

SEQ ID NO: 263 - RNA, 19 nt, synthetic construct
  source 1..19: mol_type = other RNA
tatctggccatgtcctccg

SEQ ID NO: 264 - RNA, 19 nt, synthetic construct
  source 1..19: mol_type = other RNA
ttgcagggtcttcaagccg

SEQ ID NO: 265 - RNA, 19 nt, synthetic construct
  source 1..19: mol_type = other RNA
tacacgatgaaatatgggc

SEQ ID NO: 266 - RNA, 19 nt, synthetic construct
  source 1..19: mol_type = other RNA
tcgttttccatatctctgc

SEQ ID NO: 267 - RNA, 19 nt, synthetic construct
  source 1..19: mol_type = other RNA
aaataggaaaaggccagag

SEQ ID NO: 268 - RNA, 19 nt, synthetic construct
  source 1..19: mol_type = other RNA
agagcggagtagtatctgg

SEQ ID NO: 269 - RNA, 19 nt, synthetic construct
  source 1..19: mol_type = other RNA
tgatgtagtgtcgcagcgc

SEQ ID NO: 270 - RNA, 19 nt, synthetic construct
  source 1..19: mol_type = other RNA
tgacaaaggaaaacattgc

SEQ ID NO: 271 - RNA, 19 nt, synthetic construct
  source 1..19: mol_type = other RNA
tcttcaagccgagttctgg

SEQ ID NO: 272 - RNA, 19 nt, synthetic construct
  source 1..19: mol_type = other RNA
tctgggaacattttctgtg

SEQ ID NO: 273 - RNA, 19 nt, synthetic construct
  source 1..19: mol_type = other RNA
tctcatttcccatcaccac

SEQ ID NO: 274 - RNA, 19 nt, synthetic construct
  source 1..19: mol_type = other RNA
tctctgcctggtgatgagg

SEQ ID NO: 275 - RNA, 19 nt, synthetic construct
  source 1..19: mol_type = other RNA
taggatgggtggattctcg

SEQ ID NO: 276 - RNA, 19 nt, synthetic construct
  source 1..19: mol_type = other RNA
tctctcatcaagaggtctg

SEQ ID NO: 277 - RNA, 19 nt, synthetic construct
  source 1..19: mol_type = other RNA
atgaggttgatgtagtgtc

SEQ ID NO: 278 - RNA, 19 nt, synthetic construct
  source 1..19: mol_type = other RNA
ttgatgtagtgtcgcagcg

SEQ ID NO: 279 - RNA, 19 nt, synthetic construct
  source 1..19: mol_type = other RNA
acaaaggaaaacattgcag

SEQ ID NO: 280 - RNA, 19 nt, synthetic construct
  source 1..19: mol_type = other RNA
attgcagggtcttcaagcc

SEQ ID NO: 281 - RNA, 19 nt, synthetic construct
  source 1..19: mol_type = other RNA
tttctctcatcaagaggtc

SEQ ID NO: 282 - RNA, 19 nt, synthetic construct
  source 1..19: mol_type = other RNA
ttttccatatctctgcctg

SEQ ID NO: 283 - RNA, 19 nt, synthetic construct
  source 1..19: mol_type = other RNA
agggtcagtccggacagcc

SEQ ID NO: 284 - RNA, 19 nt, synthetic construct
  source 1..19: mol_type = other RNA
acattttctgtgctttctc

SEQ ID NO: 285 - RNA, 19 nt, synthetic construct
  source 1..19: mol_type = other RNA
aatatgggctgaaaatagg

SEQ ID NO: 286 - RNA, 19 nt, synthetic construct
  source 1..19: mol_type = other RNA
acagggcgagggtcagtcc

SEQ ID NO: 287 - RNA, 19 nt, synthetic construct
  source 1..19: mol_type = other RNA
acacgagcagggacagggc

SEQ ID NO: 288 - RNA, 19 nt, synthetic construct
  source 1..19: mol_type = other RNA
attctcgttttacacgatg

SEQ ID NO: 289 - RNA, 19 nt, synthetic construct
  source 1..19: mol_type = other RNA
tggccatgtcctccgctgg

SEQ ID NO: 290 - RNA, 19 nt, synthetic construct
  source 1..19: mol_type = other RNA
ttttacacgatgaaatatg

SEQ ID NO: 291 - RNA, 19 nt, synthetic construct
  source 1..19: mol_type = other RNA
agtagtatctggccatgtc

SEQ ID NO: 292 - RNA, 19 nt, synthetic construct
  source 1..19: mol_type = other RNA
tgaggttgatgtagtgtcg

SEQ ID NO: 293 - DNA, 22 bp, synthetic construct
  source 1..22: mol_type = other DNA
tctgtgatgcccttagatgtcc

SEQ ID NO: 294 - DNA, 20 bp, synthetic construct
  source 1..20: mol_type = other DNA
ccatccaatcggtagtagcg

SEQ ID NO: 295 - DNA, 26 bp, synthetic construct
  source 1..26: mol_type = other DNA
gcctgtgatgctgggcacttcatctg

SEQ ID NO: 296 - DNA, 26 bp, synthetic construct
  source 1..26: mol_type = other DNA
tttggttcggcagcttgctaggtgac

SEQ ID NO: 297 - DNA, 20 bp, synthetic construct
  source 1..20: mol_type = other DNA
tggccagatactactccgct

SEQ ID NO: 298 - DNA, 20 bp, synthetic construct
  source 1..20: mol_type = other DNA
gcagactggtttcaggggat

SEQ ID NO: 299 - DNA, 21 bp, synthetic construct
  source 1..21: mol_type = other DNA
gctaggtaacaagcgactggg

SEQ ID NO: 300 - DNA, 20 bp, synthetic construct
  source 1..20: mol_type = other DNA
tgggctggatcgttttccat

SEQ ID NO: 301 - DNA, 20 bp, synthetic construct
  source 1..20: mol_type = other DNA
cacctgcaaccacaatctgc

SEQ ID NO: 302 - DNA, 20 bp, synthetic construct
  source 1..20: mol_type = other DNA
gacgtcttggacacatccgt

SEQ ID NO: 303 - DNA, 19 bp, synthetic construct
  source 1..19: mol_type = other DNA
aatgcttccccgaggtgtg

SEQ ID NO: 304 - DNA, 20 bp, synthetic construct
  source 1..20: mol_type = other DNA
tggggaagatccgctggtat

SEQ ID NO: 305 - DNA, 20 bp, synthetic construct
  source 1..20: mol_type = other DNA
ggatctgcatcaggcacact

SEQ ID NO: 306 - DNA, 20 bp, synthetic construct
  source 1..20: mol_type = other DNA
cgccttaggtagcaagccat

SEQ ID NO: 307 - DNA, 21 bp, synthetic construct
  source 1..21: mol_type = other DNA
ctccctcgccaccaaaacttc

SEQ ID NO: 308 - DNA, 22 bp, synthetic construct
  source 1..22: mol_type = other DNA
gtgaaggtgggaggatcagaga

SEQ ID NO: 309 - DNA, 20 bp, synthetic construct
  source 1..20: mol_type = other DNA
ggtacagcaagaagacggca

SEQ ID NO: 310 - DNA, 20 bp, synthetic construct
  source 1..20: mol_type = other DNA
ttctcgtgagggaacgcttg

SEQ ID NO: 311 - DNA, 20 bp, synthetic construct
  source 1..20: mol_type = other DNA
aatactgctgccactcggaa

SEQ ID NO: 312 - DNA, 20 bp, synthetic construct
  source 1..20: mol_type = other DNA
ggccagattgcctatgagga

SEQ ID NO: 313 - DNA, 26 bp, synthetic construct
  source 1..26: mol_type = other DNA
gagatggcagggactctgataacacc

SEQ ID NO: 314 - DNA, 26 bp, synthetic construct
  source 1..26: mol_type = other DNA
aaagtgctaggattacaggcgtgagc

SEQ ID NO: 315 - DNA, 19 bp, synthetic construct
  source 1..19: mol_type = other DNA
aggagacggaatacagggc

SEQ ID NO: 316 - DNA, 20 bp, synthetic construct
  source 1..20: mol_type = other DNA
ccacgtagtagacgatgggc

SEQ ID NO: 317 - DNA, 20 bp, synthetic construct
  source 1..20: mol_type = other DNA
agccccttgagactacgggt

SEQ ID NO: 318 - DNA, 20 bp, synthetic construct
  source 1..20: mol_type = other DNA
cgtcaatgggaacctgtgcg

SEQ ID NO: 319 - DNA, 21 bp, synthetic construct
  source 1..21: mol_type = other DNA
ccagccatctttcattgggat

SEQ ID NO: 320 - DNA, 20 bp, synthetic construct
  source 1..20: mol_type = other DNA
cccctgacaggacgttgtta

SEQ ID NO: 321 - RNA, 19 nt, synthetic construct
  source 1..19: mol_type = other RNA
aaatcgcgagacgcgtaca

SEQ ID NO: 322 - RNA, 19 nt, synthetic construct
  source 1..19: mol_type = other RNA
aacgatcgtaccgcgtata

SEQ ID NO: 323 - RNA, 19 nt, synthetic construct
  source 1..19: mol_type = other RNA
acgatcgctattacgcgaa

SEQ ID NO: 324 - RNA, 19 nt, synthetic construct
  source 1..19: mol_type = other RNA
atcgtcgaaactacgccga

SEQ ID NO: 325 - RNA, 19 nt, synthetic construct
  source 1..19: mol_type = other RNA
atacgcgaaccttacgcga

SEQ ID NO: 326 - RNA, 19 nt, synthetic construct
  source 1..19: mol_type = other RNA
atacgcgctaaaatcgcga

SEQ ID NO: 327 - RNA, 19 nt, synthetic construct
  source 1..19: mol_type = other RNA
acgtagcgtatatacgcga

SEQ ID NO: 328 - RNA, 19 nt, synthetic construct
  source 1..19: mol_type = other RNA
attacgcgcgttcgcgaaa

SEQ ID NO: 329 - RNA, 19 nt, synthetic construct
  source 1..19: mol_type = other RNA
acggtacgatacgatacga

SEQ ID NO: 330 - RNA, 19 nt, synthetic construct
  source 1..19: mol_type = other RNA
acgcgataacgcgcgataa

SEQ ID NO: 331 - RNA, 19 nt, synthetic construct
  source 1..19: mol_type = other RNA
agatcgcgtacctacgaga

SEQ ID NO: 332 - RNA, 19 nt, synthetic construct
  source 1..19: mol_type = other RNA
attgcgctatcgagtacga

SEQ ID NO: 333 - RNA, 19 nt, synthetic construct
  source 1..19: mol_type = other RNA
agcgttacggtatcgcaaa

SEQ ID NO: 334 - RNA, 19 nt, synthetic construct
  source 1..19: mol_type = other RNA
atacgacatgccttacgca

SEQ ID NO: 335 - RNA, 19 nt, synthetic construct
  source 1..19: mol_type = other RNA
aacggcgaactgccgataa

SEQ ID NO: 336 - RNA, 19 nt, synthetic construct
  source 1..19: mol_type = other RNA
agcgatagatgtcgcgcta

SEQ ID NO: 337 - RNA, 19 nt, synthetic construct
  source 1..19: mol_type = other RNA
aaacgcgctgatacgacga

SEQ ID NO: 338 - RNA, 19 nt, synthetic construct
  source 1..19: mol_type = other RNA
acgaacgcagtttcgcgta

SEQ ID NO: 339 - RNA, 19 nt, synthetic construct
  source 1..19: mol_type = other RNA
acgcgatagctatcgtcga

SEQ ID NO: 340 - RNA, 19 nt, synthetic construct
  source 1..19: mol_type = other RNA
acgatcgcgtattacgcga

SEQ ID NO: 341 - RNA, 19 nt, synthetic construct
  source 1..19: mol_type = other RNA
acgcgtaacattatcgcga

SEQ ID NO: 342 - RNA, 19 nt, synthetic construct
  source 1..19: mol_type = other RNA
aatacgcgtagcgcgttaa

SEQ ID NO: 343 - RNA, 19 nt, synthetic construct
  source 1..19: mol_type = other RNA
acgcgttacctatacgcga

SEQ ID NO: 344 - RNA, 19 nt, synthetic construct
  source 1..19: mol_type = other RNA
acgttacgtgatcgcgtaa

SEQ ID NO: 345 - RNA, 19 nt, synthetic construct
  source 1..19: mol_type = other RNA
attacgcgacgcgcgataa

SEQ ID NO: 346 - RNA, 19 nt, synthetic construct
  source 1..19: mol_type = other RNA
agtacgcactagtacgtaa

SEQ ID NO: 347 - RNA, 19 nt, synthetic construct
  source 1..19: mol_type = other RNA
actacgcaaccggcgtata

SEQ ID NO: 348 - RNA, 19 nt, synthetic construct
  source 1..19: mol_type = other RNA
attacgctatgcacgcgaa

SEQ ID NO: 349 - RNA, 19 nt, synthetic construct
  source 1..19: mol_type = other RNA
atcgcgattaggtcgcgta

SEQ ID NO: 350 - RNA, 19 nt, synthetic construct
  source 1..19: mol_type = other RNA
atacgcgttcagcgtacga